European Patent Specification EP 4 247 973 B1, published April 8, 2026. Title: DETECTING METHYLATION CHANGES IN DNA SAMPLES USING RESTRICTION ENZYMES AND HIGH THROUGHPUT SEQUENCING. Applicant: NUCLEIX LTD. The sequence listing filed with the application follows.

SEQUENCE LISTING (6 sequences)

SEQ ID NO: 1 - DNA, 85 bp, Homo sapiens
agtagcgcccactgagcggtttttcagttgctgcaccgttcttagcgcccaacggaacgtttcccgtacgcggagtccataagtt

SEQ ID NO: 2 - DNA, 69 bp, Homo sapiens
cggtcccgcagcgcccgccacacacccgcgccagaggtccagcgcatgtgcagtgaaatggcctagccc

SEQ ID NO: 3 - DNA, 72 bp, Homo sapiens
cggatagcgcggcgggcgacagccccccggataaccccgccgagggaggggcgcttgtaaaaccgagcggcg

SEQ ID NO: 4 - DNA, 60 bp, Homo sapiens
tcctccttgccttctttcgccgaaagggggcgcgctcctcccaggctgcgctggtaccta

SEQ ID NO: 5 - DNA, 78 bp, Homo sapiens
aggacccgctccgcaaagcgcccaccctcgagggaggaaagccgagctgcgcctccgcgcaaggccagggagtgtggc

SEQ ID NO: 6 - DNA, 73 bp, Homo sapiens
aggccgcgagcgcggcgcgatcagtagcgcccactaacagttcgttctgcacggcggagcgcgagaccgcgga